European Patent Specification EP 3 467 113 B1, published June 7, 2023. Title: method for production of alfa-hydromuconate. Applicant: Toray Industries, Inc. The sequence listing filed with the application follows.

SEQUENCE LISTING (12 sequences)

SEQ ID NO: 1 - DNA, 200 bp, Escherichia coli
  5'UTR (1)..(200)
cgtaattgccctttaaaattcggggcgccgaccccatgtggtctcaagcccaaaggaagagtgaggcgagtcagtcgcgtaatgcttaggcacaggattgatttgtcgcaatgattgacacgattccgcttgacgctgcgtaaggtttttgtaattttacaggcaaccttttattcactaacaaatagctggtggaatat

SEQ ID NO: 2 - DNA, 30 bp, Artificial Sequence
  Artificial Sequence
  primer (1)..(30)
taccgtcgacctcgacgtaattgcccttta

SEQ ID NO: 3 - DNA, 41 bp, Artificial Sequence
  Artificial Sequence
  primer (1)..(41)
ggccccccctcgagtcattaagtactatattccaccagcta

SEQ ID NO: 4 - DNA, 1203 bp, Serratia plymuthica
  gene (1)..(1203)
atgaatccagcctatctgtgtgacgccgttcgtacgccttttggccgtctgaacggcagtctcgccactgtccgcgccgacgatctggccgccctgccgctgaaagcgctacaggcgcgccacccgcagcttgactggagcgcggtagacgacgtgttgctcggctgcgccaaccaggcgggagaagataaccgcaacgtagcacgcatggcgctgctgctggccggcctgccggtgcagatccccggttgcaccctcaatcgtctgtgcggctccagcctggatgctgtggcgatggcggcccgcgccatcaagacaggtgaaagtgagctgatgattgccggtggcgtggaaagcatgtcgcgggcgccgtttgtgatgggcaaagcggagagcgcctttagccgggcgatgaaaatagaagacaccaccatgggctggcggtttatcaatccgcaaatgcaggcgcaatacggcgtggactctatgccgcagaccgctgaaaacgtagccctgaagtttggcattagccgccaggatcaggatgctttcgccctgcgcagccagcaacgcaccgcagcggcccaggaaagcggtttctttgccgagcaactgatcgaagtcagtctggcgcagaaaaaaggcgacccactgctgttccgccaggatgaacatccgcgcgccactacgctcgaggcactggcgaagttgaaaccggtagttaatccgcaaggtaccgtcaccgccggtaatgcctccgggctgaacgacggtgcctgcgcactgttgctggccggagagcgcggagtaacccgccacggcttggagccaatggcgcgcattgtcgccagcgccgtgaccggcattgaaccttcgattatgggctttgcgccgacagaggcggtgcgcaaagtgctgaaaatcgccggtctgacgctcgatcaaatggacgttatcgaacttaacgaagcctttgcagcgcaggcgctggcggtgactcgtgagctgggactgagtgacgacgccgcacaggtgaacccaaacggcggcgcgattgcgctgggccatccgctgggtgcttccggtggcaggctggtgatgaacgccgcctggcaattgcagaaaacacggggacgctacgggttatgcaccatgtgcatcggcgttggccaaggtattgcgctgatcatcgagcgggtatga

SEQ ID NO: 5 - DNA, 30 bp, Artificial Sequence
  Artificial Sequence
  primer (1)..(30)
ctggtggaatatagtatgaatccagcctat

SEQ ID NO: 6 - DNA, 30 bp, Artificial Sequence
  Artificial Sequence
  primer (1)..(30)
ctcgagtcattaagttcatacccgctcgat

SEQ ID NO: 7 - DNA, 53 bp, Artificial Sequence
  Artificial Sequence
  primer (1)..(53)
ctggtggaatatagtacttagctggtggaatatatgaaccctcaagatattgt

SEQ ID NO: 8 - DNA, 41 bp, Artificial Sequence
  Artificial Sequence
  primer (1)..(41)
ctcgagtcattaagtgttaacttagttctccttttcaaaga

SEQ ID NO: 9 - DNA, 30 bp, Artificial Sequence
  Artificial Sequence
  primer (1)..(30)
caagagtccggatccatgatgataaatgtg

SEQ ID NO: 10 - DNA, 34 bp, Artificial Sequence
  Artificial Sequence
  primer (1)..(34)
cgagctcccaattgggatcagatctttatgactc

SEQ ID NO: 11 - DNA, 35 bp, Artificial Sequence
  Artificial Sequence
  Primer (1)..(35)
cggatcccaattgggagctcatgaatccagcctat

SEQ ID NO: 12 - DNA, 35 bp, Artificial Sequence
  Artificial Sequence
  Primer (1)..(35)
gcgccgtgtacacgagatcttcatacccgctcgat